European Patent Specification EP 3 728 283 B1, published November 22, 2023. Title: 3'3' CYCLIC DINUCLEOTIDES WITH PHOSPHONATE BOND ACTIVATING THE STING ADAPTOR PROTEIN. Applicant: Birkus, Gabriel Pav, Ondrej Jandusik, Tomas Rosenberg, Ivan Nencka, Radim. The sequence listing filed with the application follows.

SEQUENCE LISTING (12 sequences)

SEQ ID NO: 1 - DNA, 75 bp, Artificial Sequence
  Synthetic construct
aaagatcttggaaagtgaaaccttggaaaacgaaactggacaaagggaaactgcagaaactgaaacaaagcttaa

SEQ ID NO: 2 - DNA, 75 bp, Artificial Sequence
  Synthetic construct
ttaagctttgtttcagtttctgcagtttccctttgtccagtttcgttttccaaggtttcactttccaagatcttt

SEQ ID NO: 3 - DNA, 20 bp, Artificial Sequence
  Synthetic construct
tgcttgctcaactctacgtc

SEQ ID NO: 4 - DNA, 20 bp, Artificial Sequence
  Synthetic construct
gtggtttgtccaaactcatc

SEQ ID NO: 5 - DNA, 31 bp, Artificial Sequence
  Synthetic construct
gtgggatccgccccagctgagatctctgcag

SEQ ID NO: 6 - DNA, 38 bp, Artificial Sequence
  Synthetic construct
tatgcggccgcctattacacagtaacctcttccttttc

SEQ ID NO: 7 - DNA, 330 bp, Artificial Sequence
  Synthetic construct
atgtcgcatcaccatcatcatcaccaccatgggatgtcggactcagaagtcaatcaagaagctaagccagaggtcaagccagaagtcaagcctgagactcacatcaatttaaaggtgtccgatggatcttcagagatcttcttcaagatcaaaaagaccactcctttaagaaggctgatggaagcgttcgctaaaagacagggtaaggaaatggactccttaagattcttgtacgacggtattagaattcaagctgatcagacccctgaagatttggacatggaggataacgatattattgaggctcaccgcgaacagattggtggatcc

SEQ ID NO: 8 - protein, 110 aa, Artificial Sequence
  Synthetic construct
MSHHHHHHHHGMSDSEVNQEAKPEVKPEVKPETHINLKVSDGSSEIFFKIKKTTPLRRLMEAFAKRQGKEMDSLRFLYDGIRIQADQTPEDLDMEDNDIIEAHREQIGGS

SEQ ID NO: 9 - protein, 204 aa, Artificial Sequence
  Synthetic construct
APAEISAVCEKGNFNVAHGLAWSYYIGYLRLILPELQARIRTYNQHYNNLLRGAVSQRLYILLPLDCGVPDNLSMADPNIRFLDKLPQQTGDRAGIKDRVYSNSIYELLENGQRAGTCVLEYATPLQTLFAMSQYSQAGFSREDRLEQAKLFCRTLEDILADAPESQNNCRLIAYQEPADDSSFSLSQEVLRHLRQEEKEEVTV

SEQ ID NO: 10 - protein, 204 aa, Artificial Sequence
  Synthetic construct
APAEISAVCEKGNFNVAHGLAWSYYIGYLRLILPELQARIRTYNQHYNNLLRGAVSQRLYILLPLDCGVPDNLSMADPNIRFLDKLPQQTADRAGIKDRVYSNSIYELLENGQRAGTCVLEYATPLQTLFAMSQYSQAGFSREDRLEQAKLFCQTLEDILADAPESQNNCRLIAYQEPADDSSFSLSQEVLRHLRQEEKEEVTV

SEQ ID NO: 11 - protein, 502 aa, Artificial Sequence
  Synthetic construct
MNSSHHHHHHMQYKLILNGKTLKGETTTEAVDAATAEKVLKQYANDNGVDGEWTYDDATKTFTVTENNNNNNNNNNENLYFQGMRMTWNFHQYYTNRNDGLMGKLVLTDEEKNNLKALRKIIRLRTRDVFEEAKGIAKAVKKSALTFEIIQEKVSTTQIKHLSDSEQREVAKLIYEMDDDARDEFLGLTPRFWTQGSFQYDTLNRPFQPGQEMDIDDGTYMPMPIFESEPKIGHSLLILLVDASLKSLVAENHGWKFEAKQTCGRIKIEAEKTHIDVPMYAIPKDEFQKKQIALEANRSFVKGAIFESYVADSITDDSETYELDSENVNLALREGDRKWINSDPKIVEDWFNDSCIRIGKHLRKVCRFMKAWRDAQWDVGGPSSISLMAATVNILDSVAHDASDLGETMKIIAKHLPSEFARGVESPDSTDEKPLFPPSYKHGPREMDIMSKLERLPEILSSAESADSKSEALKKINMAFGNRVTNSELIVLAKALPAFAQE

SEQ ID NO: 12 - protein, 365 aa, Artificial sequence
  Synthetic polypeptide
MEENKQRVKSMINILQLVAPGTPLREGIDNVLRAQTGGLIVLGYNEQIKSIVDGGFHINCAFSPASLYELAKMDGALILNETGSKILIANAQLVPDSSIDSIETGMRHRTAERVAKQTGSLVVAISQRRNVITLYQGNLRYTLKDIGVILTKANQAIQTLEKYKAVWNDGITNLGILEFEEVVTMSEVVHVLHSVEMVLRIKNEILSYIHELGTEGRLIRLQLTELLADLEAEAALLIKDYHQEKTQDHHQILKKLQDLANTQLLEDSDLVKLLGYPGQTSLEESVTPRGYRITSKISRVPPLIIENLINRFKTLQGVCRATINELDDVEGIGEVRAKKIREGLKRIQEHLYMSRHNLEHHHHHH